European Patent Application EP 4 790 148 A1, published August 12, 2026. Title: DNA甲基化标志物TAGMe-7的鉴定及其在肿瘤检测中的用途. Applicant: 上海奕谱生物科技有限公司. Application CN. The sequence listing filed with the application follows.

SEQUENCE LISTING (30 sequences)

SEQ ID NO: 1 - DNA, 1006 bp, Homo sapiens
  source 1..1006: mol_type = genomic DNA
cagtggccggatggaagtagcgaagggcgacgaagccgcggccgccgcgcctgaggctgcagccgcggccgccgccgccgtgacgcccacgtgcgggtagtagtgcagcggcacgtgcgagtggaaggggtagggcaggcttccggtggcggccgcgtgcgtcatcatgtaggtgtagaagctggggtcggctgggtgcggccaggacatggccaggcgctgccgcttgtccttcatgcgccggttctggaaccacacctgcggggagagacgcgccgcagcctgggttagggagcgccccgtgttcccagctcctgtcccaggacctctgccccttccggacctctgaatggcttggtctacttctctccgaccaagcccaaccccgagtaccctgtggtctcccagctgggaaagtgtggacggcagtgtgtggaccgccgtgggcacaccgtcctcaacgaagagggtcctctcccccgcgtccggctgctgctgctcctcaggcttttattcccttacttcttgctgcacttttttgtcccaatccaacctttcctctccctcccgccacccaccagtgccggtctcgctgagcacccgtctctcaatcccaggatttgtacggggattctgggcagcctttgaagagaggctgccgctcagcttttctgagaggtcgccgcgcgaagtcttgagccctccgaactgcaaggacctgcccctaggggcacgggtccgattttgatattgaagggatgattttgttggaatcgtttgccttaaatgagtgggtagagcaatgtctccataaacggggaaggggacgtttccacccctcccaacactatctaataaagacatcattcgtcacaactctaaattaaagaaagcccgatcaaaccagagggagacttccacactcctcccctaccccgtggagattttttcttttttctgcagtgtcgaacgctccatgaagggctcaccaaatcgcctaacctcc

SEQ ID NO: 2 - DNA, 1006 bp, synthetic construct
  source 1..1006: mol_type = other DNA
tagtggtyggatggaagtagygaagggygaygaagtygyggtygtygygtttgaggttgtagtygyggtygtygtygtygtgaygtttaygtgygggtagtagtgtagyggtaygtgygagtggaaggggtagggtaggttttyggtggyggtygygtgygttattatgtaggtgtagaagttggggtyggttgggtgyggttaggatatggttaggygttgtygtttgttttttatgygtyggttttggaattatatttgyggggagagaygygtygtagtttgggttagggagygtttygtgtttttagtttttgttttaggatttttgtttttttyggatttttgaatggtttggtttattttttttygattaagtttaatttygagtattttgtggttttttagttgggaaagtgtggayggtagtgtgtggatygtygtgggtatatygtttttaaygaagagggttttttttttygygttyggttgttgttgttttttaggtttttatttttttattttttgttgtatttttttgttttaatttaattttttttttttttttygttatttattagtgtyggtttygttgagtattygttttttaattttaggatttgtayggggattttgggtagtttttgaagagaggttgtygtttagtttttttgagaggtygtygygygaagttttgagtttttygaattgtaaggatttgtttttaggggtaygggttygattttgatattgaagggatgattttgttggaatygtttgttttaaatgagtgggtagagtaatgtttttataaayggggaaggggaygtttttattttttttaatattatttaataaagatattattygttataattttaaattaaagaaagttygattaaattagagggagatttttatattttttttttatttygtggagatttttttttttttttgtagtgtygaaygttttatgaagggtttattaaatygtttaattttt

SEQ ID NO: 3 - DNA, 1006 bp, synthetic construct; identical to SEQ ID NO: 2
  source 1..1006: mol_type = other DNA

SEQ ID NO: 4 - DNA, 57 bp, synthetic construct
  source 1..57: mol_type = other DNA
gacgtgtgctcttccgatcttagcttractttcccaactaaaaaaccacaaaatact

SEQ ID NO: 5 - DNA, 58 bp, synthetic construct
  source 1..58: mol_type = other DNA
aatgatacggcgaccaccgagatctacactctttccctacacgacgctcttccgatct

SEQ ID NO: 6 - DNA, 64 bp, synthetic construct
  source 1..64: mol_type = other DNA
caagcagaagacggcatacgagatcgtgatgtgactggagttcagacgtgtgctcttccgatct

SEQ ID NO: 7 - DNA, 28 bp, synthetic construct
  source 1..28: mol_type = other DNA
tacacgacgctcttccgatctcgtgaty

SEQ ID NO: 8 - DNA, 28 bp, synthetic construct
  source 1..28: mol_type = other DNA
tacacgacgctcttccgatctacatcgy

SEQ ID NO: 9 - DNA, 28 bp, synthetic construct
  source 1..28: mol_type = other DNA
tacacgacgctcttccgatctgcctaay

SEQ ID NO: 10 - DNA, 28 bp, synthetic construct
  source 1..28: mol_type = other DNA
tacacgacgctcttccgatcttggtcay

SEQ ID NO: 11 - DNA, 28 bp, synthetic construct
  source 1..28: mol_type = other DNA
tacacgacgctcttccgatctcactgty

SEQ ID NO: 12 - DNA, 28 bp, synthetic construct
  source 1..28: mol_type = other DNA
tacacgacgctcttccgatctattggcy

SEQ ID NO: 13 - DNA, 28 bp, synthetic construct
  source 1..28: mol_type = other DNA
tacacgacgctcttccgatctgatctgy

SEQ ID NO: 14 - DNA, 28 bp, synthetic construct
  source 1..28: mol_type = other DNA
tacacgacgctcttccgatcttcaagty

SEQ ID NO: 15 - DNA, 28 bp, synthetic construct
  source 1..28: mol_type = other DNA
tacacgacgctcttccgatctctgatcy

SEQ ID NO: 16 - DNA, 28 bp, synthetic construct
  source 1..28: mol_type = other DNA
tacacgacgctcttccgatctaagctay

SEQ ID NO: 17 - DNA, 27 bp, synthetic construct
  source 1..27: mol_type = other DNA
gacgtgtgctcttccgatcttagcttr

SEQ ID NO: 18 - DNA, 27 bp, synthetic construct
  source 1..27: mol_type = other DNA
gacgtgtgctcttccgatctggctacr

SEQ ID NO: 19 - DNA, 27 bp, synthetic construct
  source 1..27: mol_type = other DNA
gacgtgtgctcttccgatctcttgtar

SEQ ID NO: 20 - DNA, 27 bp, synthetic construct
  source 1..27: mol_type = other DNA
gacgtgtgctcttccgatctagtcaar

SEQ ID NO: 21 - DNA, 27 bp, synthetic construct
  source 1..27: mol_type = other DNA
gacgtgtgctcttccgatctagttccr

SEQ ID NO: 22 - DNA, 27 bp, synthetic construct
  source 1..27: mol_type = other DNA
gacgtgtgctcttccgatctccgaccr

SEQ ID NO: 23 - DNA, 27 bp, synthetic construct
  source 1..27: mol_type = other DNA
gacgtgtgctcttccgatctggacggr

SEQ ID NO: 24 - DNA, 27 bp, synthetic construct
  source 1..27: mol_type = other DNA
gacgtgtgctcttccgatctctctacr

SEQ ID NO: 25 - DNA, 27 bp, synthetic construct
  source 1..27: mol_type = other DNA
gacgtgtgctcttccgatctgcggacr

SEQ ID NO: 26 - DNA, 27 bp, synthetic construct
  source 1..27: mol_type = other DNA
gacgtgtgctcttccgatcttgtgatr

SEQ ID NO: 27 - DNA, 25 bp, synthetic construct
  source 1..25: mol_type = other DNA
tagtggtyggatggaagtagygaag

SEQ ID NO: 28 - DNA, 25 bp, synthetic construct
  source 1..25: mol_type = other DNA
ctccccrcaaatataattccaaaac

SEQ ID NO: 29 - DNA, 25 bp, synthetic construct
  source 1..25: mol_type = other DNA
gtggttttttagttgggaaagtgtg

SEQ ID NO: 30 - DNA, 25 bp, synthetic construct
  source 1..25: mol_type = other DNA
aattaaacratttaataaacccttc